European Patent Application EP 4 667 489 A1, published December 24, 2025. Title: 一种多肽以及包含其作为轻链的抗体. Applicant: 康源博创生物科技（北京）有限公司. The sequence listing filed with the application follows.

SEQUENCE LISTING (56 sequences)

SEQ ID NO: 1 - protein, 105 aa, synthetic construct
QIVLTQSPAIMSASPGEKVTMTCSASSSVSYMHWYQQKSGTSPKRWIYDTSKLASGVPARFSGSGSGTSYSLTISSMEAEDAATYYCQQWSSNPPFGSGTKLEIK

SEQ ID NO: 2 - protein, 107 aa, synthetic construct
QIVLTQSPAIMSASPGEKVTMTCSASSSVSYMHWYQQKSGTSPKRWIYDTSKLASGVPARFSGSGSGTSYSLTISSMEAEDAATYYCQQWSSNPPYTFGSGTKLEIK

SEQ ID NO: 3 - protein, 107 aa, synthetic construct
QIVLTQSPAIMSASPGEKVTMTCSASSSVSYMHWYQQKSGTSPKRWIYDTSKLASGVPARFSGSGSGTSYSLTISSMEAEDAATYYCQQWSSNPPWTFGSGTKLEIK

SEQ ID NO: 4 - protein, 107 aa, synthetic construct
QIVLTQSPAIMSASPGEKVTMTCSASSSVSYMHWYQQKSGTSPKRWIYDTSKLASGVPARFSGSGSGTSYSLTISSMEAEDAATYYCQQWSSNPPFTFGSGTKLEIK

SEQ ID NO: 5 - protein, 120 aa, synthetic construct
LDVKLQESGPGLVKPSQSLSLTCSVTGYSFTSGYYWNWIRLFPGNKLEWMGYVSYFGTNNYNPSLKNRFSITRDTSKNQFFLKLNSVSTEDTATYYCARGEEWDWSFDVWGTGTTVTVSS

SEQ ID NO: 6 - RNA, 20 nt, synthetic construct
  source 1..20: mol_type = other RNA
tgaatgccatgtacttatgg

SEQ ID NO: 7 - RNA, 20 nt, synthetic construct
  source 1..20: mol_type = other RNA
aagttcagctcctaaaatgg

SEQ ID NO: 8 - RNA, 21 nt, synthetic construct
  source 1..21: mol_type = other RNA
gtgaatgccatgtacttatgg

SEQ ID NO: 9 - RNA, 21 nt, synthetic construct
  source 1..21: mol_type = other RNA
caagttcagctcctaaaatgg

SEQ ID NO: 10 - protein, 119 aa, synthetic construct
DVKLQESGPGLVKPSQSLSLTCSVTGYSFTSGYYWNWIRLFPGNKLEWMGYVSYFGTNNYNPSLKNRFSITRDTSKNQFFLKLNSVSTEDTATYYCARGEEWDWSFDVWGTGTTVTVSS

SEQ ID NO: 11 - protein, 107 aa, synthetic construct
DIVLTQSPAFMSASPGEKVTMTCSASSSVSYMHWYQQKSGTSPKRWIYDTSKLASGVPTRFSGSGSGTSYSLTISSMEAEDAATYYCQQWSTNPPYTFGGGTKLEIK

SEQ ID NO: 12 - protein, 122 aa, synthetic construct
QVQLKESGGGLVKPGGSLKLSCAASGFTFSDYGMHWVRQAPEKGLEWVAYISSGSYTIYYADTVRDRFTISRDSAKNTLFLQMTSLRSEDTAMYYCVRRGPGYFGSTALDYWGQGTTLTVSS

SEQ ID NO: 13 - protein, 107 aa, synthetic construct
QIVLTQSPAIMSASPGEKVTMTCSATSGVSYMHWYQQKSGTSPKRWIYDTSRLASGVPARFSGSGSGTSYSLTISSMEAEDAATYYCQQWSSNPPYTFGSGTKLEIK

SEQ ID NO: 14 - protein, 122 aa, synthetic construct
QVQLVESGGGLVKPGGSLRLSCAASGFTFSDYGMHWIRQAPGKGLEWVAYISSGSYTIYYADTVRDRFTISRDSAKNSLYLQMNSLRAEDTAVYYCVRRGPGYFGSTALDYWGQGTTVTVSS

SEQ ID NO: 15 - protein, 107 aa, synthetic construct
DIQITQSPSSLSASVGDRVTITCSATSGVSYMHWYQQKPGKAPKRLIYDTSRLASGVPSRFSGSGSGTDYTLTISSLQPEDFATYYCQQWSSNPPYTFGQGTRLEIK

SEQ ID NO: 16 - protein, 107 aa, synthetic construct
DIQITQSPSSLSASVGDRVTITCSASSSVSYMHWYQQKPGKAPKRLIYDTSKLASGVPSRFSGSGSGTDYTLTISSLQPEDFATYYCQQWSSNPPYTFGQGTRLEIK

SEQ ID NO: 17 - protein, 327 aa, synthetic construct
ASTKGPSVFPLAPCSRSTSESTAALGCLVKDYFPEPVTVSWNSGALTSGVHTFPAVLQSSGLYSLSSVVTVPSSSLGTKTYTCNVDHKPSNTKVDKRVESKYGPPCPPCPAPEFLGGPSVFLFPPKPKDTLMISRTPEVTCVVVDVSQEDPEVQFNWYVDGVEVHNAKTKPREEQFNSTYRVVSVLTVLHQDWLNGKEYKCKVSNKGLPSSIEKTISKAKGQPREPQVYTLPPSQEEMTKNQVSLTCLVKGFYPSDIAVEWESNGQPENNYKTTPPVLDSDGSFFLYSRLTVDKSRWQEGNVFSCSVMHEALHNHYTQKSLSLSLGK

SEQ ID NO: 18 - protein, 107 aa, synthetic construct [sequence omitted]

SEQ ID NO: 19 - protein, 119 aa, synthetic construct
QVQLQESGPGLVKPSETLSLTCTVSGYSFTSGYYWNWIRQPPGKGLEWIGYVSYFGTANYNPALKNRVTISRDTSKNQFSLKLSSVTAADTAVYYCARGEEWDWSFDVWGQGTTVTVSS

SEQ ID NO: 20 - protein, 326 aa, synthetic construct
ASTKGPSVFPLAPCSRSTSESTAALGCLVKDYFPEPVTVSWNSGALTSGVHTFPAVLQSSGLYSLSSVVTVPSSSLGTKTYTCNVDHKPSNTKVDKRVESKYGPPCPPCPAPEFLGGPSVFLFPPKPKDTLMISRTPEVTCVVVDVSQEDPEVQFNWYVDGVEVHNAKTKPREEQFNSTYRVVSVLTVLHQDWLNGKEYKCKVSNKGLPSSIEKTISKAKGQPREPQVYTLPPCQEEMTKNQVSLWCLVKGFYPSDIAVEWESNGQPENNYKTTPPVLDSDGSFFLYSRLTVDKSRWQEGNVFSCSVMHEALHNHYTQKSLSLSLG

SEQ ID NO: 21 - protein, 326 aa, synthetic construct
ASTKGPSVFPLAPCSRSTSESTAALGCLVKDYFPEPVTVSWNSGALTSGVHTFPAVLQSSGLYSLSSVVTVPSSSLGTKTYTCNVDHKPSNTKVDKRVESKYGPPCPPCPAPEFLGGPSVFLFPPKPKDTLMISRTPEVTCVVVDVSQEDPEVQFNWYVDGVEVHNAKTKPREEQFNSTYRVVSVLTVLHQDWLNGKEYKCKVSNKGLPSSIEKTISKAKGQPREPQVCTLPPSQEEMTKNQVSLSCAVKGFYPSDIAVEWESNGQPENNYKTTPPVLDSDGSFFLVSRLTVDKSRWQEGNVFSCSVMHEALHNHYTQKSLSLSLG

SEQ ID NO: 22 - protein, 6 aa, synthetic construct
SGYYWN

SEQ ID NO: 23 - protein, 16 aa, synthetic construct
YVSYFGTNNYNPSLKN

SEQ ID NO: 24 - protein, 10 aa, synthetic construct
GEEWDWSFDV

SEQ ID NO: 25 - protein, 10 aa, synthetic construct
SASSSVSYMH

SEQ ID NO: 26 - protein, 7 aa, synthetic construct
DTSKLAS

SEQ ID NO: 27 - protein, 10 aa, synthetic construct
QQWSTNPPYT

SEQ ID NO: 28 - protein, 5 aa, synthetic construct
DYGMH

SEQ ID NO: 29 - protein, 17 aa, synthetic construct
YISSGSYTIYYADTVRD

SEQ ID NO: 30 - protein, 13 aa, synthetic construct
RGPGYFGSTALDY

SEQ ID NO: 31 - protein, 10 aa, synthetic construct
SATSGVSYMH

SEQ ID NO: 32 - protein, 10 aa, synthetic construct
QQWSSNPPYT

SEQ ID NO: 33 - protein, 7 aa, synthetic construct
DTSRLAS

SEQ ID NO: 34 - protein, 16 aa, synthetic construct
YVSYFGTANYNPALKN

SEQ ID NO: 35 - protein, 214 aa, synthetic construct
QIVLTQSPAIMSASPGEKVTMTCSASSSVSYMHWYQQKSGTSPKRWIYDTSKLASGVPARFSGSGSGTSYSLTISSMEAEDAATYYCQQWSSNPPYTFGSGTKLEIKRTVAAPSVFIFPPSDEQLKSGTASVVCLLNNFYPREAKVQWKVDNALQSGNSQESVTEQDSKDSTYSLSSTLTLSKADYEKHKVYACEVTHQGLSSPVTKSFNRGEC

SEQ ID NO: 36 - protein, 214 aa, synthetic construct
QIVLTQSPAIMSASPGEKVTMTCSATSGVSYMHWYQQKSGTSPKRWIYDTSRLASGVPARFSGSGSGTSYSLTISSMEAEDAATYYCQQWSSNPPYTFGSGTKLEIKRTVAAPSVFIFPPSDEQLKSGTASVVCLLNNFYPREAKVQWKVDNALQSGNSQESVTEQDSKDSTYSLSSTLTLSKADYEKHKVYACEVTHQGLSSPVTKSFNRGEC

SEQ ID NO: 37 - protein, 214 aa, synthetic construct
DIQITQSPSSLSASVGDRVTITCSATSGVSYMHWYQQKPGKAPKRLIYDTSRLASGVPSRFSGSGSGTDYTLTISSLQPEDFATYYCQQWSSNPPYTFGQGTRLEIKRTVAAPSVFIFPPSDEQLKSGTASVVCLLNNFYPREAKVQWKVDNALQSGNSQESVTEQDSKDSTYSLSSTLTLSKADYEKHKVYACEVTHQGLSSPVTKSFNRGEC

SEQ ID NO: 38 - protein, 214 aa, synthetic construct
DIQITQSPSSLSASVGDRVTITCSASSSVSYMHWYQQKPGKAPKRLIYDTSKLASGVPSRFSGSGSGTDYTLTISSLQPEDFATYYCQQWSSNPPYTFGQGTRLEIKRTVAAPSVFIFPPSDEQLKSGTASVVCLLNNFYPREAKVQWKVDNALQSGNSQESVTEQDSKDSTYSLSSTLTLSKADYEKHKVYACEVTHQGLSSPVTKSFNRGEC

SEQ ID NO: 39 - protein, 121 aa, synthetic construct
QVQLKESGGGLVKPGGSLKLSCAASGFTFSDYGIHWVRQAPEKGLEWVAFISSGSSTIYYADTVKGRFTISRDNAKNTLFLQMTSLRSEDTAMYYCTRRDFYGSADAMDYWGQGTSVTVSS

SEQ ID NO: 40 - protein, 121 aa, synthetic construct
QVQLVESGGGLVKPGGSLRLSCAASGFTFSDYGIHWIRQAPGKGLEWVAFISSGSSTIYYADAVKGRFTISRDNAKNSLYLQMNSLRAEDTAVYYCTRRDFYGSADAMDYWGQGTTVTVSS

SEQ ID NO: 41 - protein, 107 aa, synthetic construct
DIQLTQSPSTLSASVGDRVTITCSATSSIGYMHWYQQKPGTSPKRWIYDTSKLASGVPSRFSGSGSGTEYTLTISSLQPDDFATYYCQLWSSDPPYTFGQGTRLEIK

SEQ ID NO: 42 - protein, 330 aa, synthetic construct [sequence omitted]

SEQ ID NO: 43 - protein, 214 aa, synthetic construct
DIQLTQSPSTLSASVGDRVTITCSATSSIGYMHWYQQKPGTSPKRWIYDTSKLASGVPSRFSGSGSGTEYTLTISSLQPDDFATYYCQLWSSDPPYTFGQGTRLEIKRTVAAPSVFIFPPSDEQLKSGTASVVCLLNNFYPREAKVQWKVDNALQSGNSQESVTEQDSKDSTYSLSSTLTLSKADYEKHKVYACEVTHQGLSSPVTKSFNRGEC

SEQ ID NO: 44 - protein, 122 aa, synthetic construct
EVQLQQSGPELVKPGASVKISCKASGYTFTDYYMNWVKQSHGKSLEWIGDINPNDGGTSYNQKFKGKATLTVDKSSSTAYMELRSLTSEDSAVYYCAREILYYVTSFYFDYWGQGTTLTVSS

SEQ ID NO: 45 - protein, 122 aa, synthetic construct
QVQLVQSGAEVKKPGASVKVSCKASGYTFTDYYMNWVRQAPGQGLEWIGDINPNDGGTSYNQKFKGRATLTVDKSTSTAYMELSSLRSEDTAVYYCAREILYYVTSFYFDYWGQGTTVTVSS

SEQ ID NO: 46 - protein, 329 aa, synthetic construct
ASTKGPSVFPLAPSSKSTSGGTAALGCLVKDYFPEPVTVSWNSGALTSGVHTFPAVLQSSGLYSLSSVVTVPSSSLGTQTYICNVNHKPSNTKVDKKVEPKSCDKTHTCPPCPAPELLGGPSVFLFPPKPKDTLMISRTPEVTCVVVDVSHEDPEVKFNWYVDGVEVHNAKTKPREEQYNSTYRVVSVLTVLHQDWLNGKEYKCKVSNKALPAPIEKTISKAKGQPREPQVYTLPPCRDELTKNQVSLWCLVKGFYPSDIAVEWESNGQPENNYKTTPPVLDSDGSFFLYSKLTVDKSRWQQGNVFSCSVMHEALHNHYTQKSLSLSPG

SEQ ID NO: 47 - protein, 329 aa, synthetic construct
ASTKGPSVFPLAPSSKSTSGGTAALGCLVKDYFPEPVTVSWNSGALTSGVHTFPAVLQSSGLYSLSSVVTVPSSSLGTQTYICNVNHKPSNTKVDKKVEPKSCDKTHTCPPCPAPELLGGPSVFLFPPKPKDTLMISRTPEVTCVVVDVSHEDPEVKFNWYVDGVEVHNAKTKPREEQYNSTYRVVSVLTVLHQDWLNGKEYKCKVSNKALPAPIEKTISKAKGQPREPQVCTLPPSRDELTKNQVSLSCAVKGFYPSDIAVEWESNGQPENNYKTTPPVLDSDGSFFLVSKLTVDKSRWQQGNVFSCSVMHEALHNHYTQKSLSLSPG

SEQ ID NO: 48 - protein, 5 aa, synthetic construct
DYGIH

SEQ ID NO: 49 - protein, 17 aa, synthetic construct
FISSGSSTIYYADTVKG

SEQ ID NO: 50 - protein, 12 aa, synthetic construct
RDFYGSADAMDY

SEQ ID NO: 51 - protein, 17 aa, synthetic construct
FISSGSSTIYYADAVKG

SEQ ID NO: 52 - protein, 10 aa, synthetic construct
SATSSIGYMH

SEQ ID NO: 53 - protein, 10 aa, synthetic construct
QLWSSDPPYT

SEQ ID NO: 54 - protein, 5 aa, synthetic construct
DYYMN

SEQ ID NO: 55 - protein, 17 aa, synthetic construct
DINPNDGGTSYNQKFKG

SEQ ID NO: 56 - protein, 13 aa, synthetic construct
EILYYVTSFYFDY